European Patent Application EP 4 516 304 A1, published March 5, 2025. Title: 抗腫瘍剤、画像生成方法、細菌、及び製造方法. Applicant: 国立大学法人北陸先端科学技術大学院大学. The sequence listing filed with the application follows.

SEQUENCE LISTING (2 sequences)

SEQ ID NO: 1 - DNA, 1411 bp, Rhodopseudomonas palustris
  source 1..1411: mol_type = genomic DNA
agcgaacgctggcggcaggcttaacacatgcaagtcgaacgggcgtagcaatacgtcagtggcagacgggtgagtaacgcgtgggaacgtaccttttggttcggaacaacacagggaaacttgtgctaataccggataagcccttacggggaaagatttatcgccgaaagatcggcccgcgtctgattagctagttggtgaggtaatggctcaccaaggcgacgatcagtagctggtctgagaggatgatcagccacattgggactgagacacggcccaaactcctacgggaggcagcagtggggaatattggacaatgggggaaaccctgatccagccatgccgcgtgagtgatgaaggccctagggttgtaaagctcttttgtgcgggaagataatgacggtaccgcaagaataagccccggctaacttcgtgccagcagccgcggtaatacgaagggggctagcgttgctcggaatcactgggcgtaaagggtgcgtaggcgggtttctaagtcagaggtgaaagcctggagctcaactccagaactgcctttgatactggaagtcttgagtatggcagaggtgagtggaactgcgagtgtagaggtgaaattcgtagatattcgcaagaacaccagtggcgaaggcggctcactgggccattactgacgctgaggcacgaaagcgtggggagcaaacaggattagataccctggtagtccacgccgtaaacgatgaatgccagccgttagtgggtttactcactagtggcgcagctaacgctttaagcattccgcctggggagtacggtcgcaagattaaaactcaaaggaattgacgggggcccgcacaagcggtggagcatgtggtttaattcgacgcaacgcgcagaaccttaccagcccttgacatgtccaggaccggtcgcagagacgcgaccttctcttcggagcctggagcacaggtgctgcatggctgtcgtcagctcgtgtcgtgagatgttgggttaagtcccgcaacgagcgcaacccccgtccttagttgctaccatttagttgagcactctaaggagactgccggtgataagccgcgaggaaggtggggatgacgtcaagtcctcatggcccttacgggctgggctacacacgtgctacaatggcggtgacaatgggaagctaaggggcgacccttcgcaaatctcaaaaagccgtctcagttcggattgggctctgcaactcgagcccatgaagttggaatcgctagtaatcgtggatcagcatgccacggtgaatacgttcccgggccttgtacacaccgcccgtcacaccatgggagttggctttacctgaagacggtgcgctaaccagcaatgggggcagccggccacggtagggtcagcgactggggtg

SEQ ID NO: 2 - DNA, 1466 bp, Proteus mirabilis
  source 1..1466: mol_type = genomic DNA
attgaacgctggcggcaggcctaacacatgcaagtcgagcggtaacaggragaaagcttgctttcttgctgacgagcggcggacgggtgagtaatgtatggggatctgcccgatagagggggataactactggaaacggtggctaataccgcataatgtctacggaccaaagcaggggctcttcggaccttgcactatcggatgaacccatatgggattagctagtaggtggggtaaaggctcacctaggcgacgatctctagctggtctgagaggatgatcagccacactgggactgagacacggcccagactcctacgggaggcagcagtggggaatattgcacaatgggcgcaagcctgatgcagccatgccgcgtgtatgaagaaggccttagggttgtaaagtactttcagcggggaggaaggtgataaggttaatacccttrtcaattgacgttacccgcagaagaagcaccggctaactccgtgccagcagccgcggtaatacggagggtgcaagcgttaatcggaattactgggcgtaaagcgcacgcaggcggtcaattaagtcagatgtgaaagccccgagcttaacttgggaattgcatctgaaactggttggctagagtcttgtagaggggggtagaattccatgtgtagcggtgaaatgcgtagagatgtggaggaataccggtggcgaaggcggccccctggacaaagactgacgctcaggtgcgaaagcgtggggagcaaacaggattagataccctggtagtccacgctgtaaacgatgtcgatttagaggttgtggtcttgaaccgtggcttctggagctaacgcgttaaatcgaccgcctggggagtacggccgcaaggttaaaactcaaatgaattgacgggggcccgcacaagcggtggagcatgtggtttaattcgatgcaacgcgaagaaccttacctactcttgacatccagcgaatcctttagagatagaggagtgccttcgggaacgctgagacaggtgctgcatggctgtcgtcagctcgtgttgtgaaatgttgggttaagtcccgcaacgagcgcaacccttatcctttgttgccagcacgtratggtgggaactcaaaggagactgccggtgataaaccggaggaaggtggggatgacgtcaagtcatcatggcccttacgagtagggctacacacgtgctacaatggcagatacaaagagaagcgacctcgcgagagcaagcggaactcataaagtctgtcgtagtccggattggagtctgcaactcgactccatgaagtcggaatcgctagtaatcgtagatcagaatgctacggtgaatacgttcccgggccttgtacacaccgcccgtcacaccatgggagtgggttgcaaaagaagtaggtagcttaaccttcgggagggcgcttaccactttgtgattcatgactggggtg